European Patent Application EP 4 640 831 A1, published October 29, 2025. Title: NUCLEIC ACID MOLECULE AND USE THEREOF. Applicant: Nanjing Curegene Technology Co., Ltd. The sequence listing filed with the application follows.

SEQUENCE LISTING (51 sequences)

SEQ ID NO: 1 - RNA, 33 nt, synthetic construct
  source 1..33: mol_type = other RNA
ggatcctggaggcttgctgaaggctgtatgctg

SEQ ID NO: 2 - RNA, 65 nt, synthetic construct
  source 1..65: mol_type = other RNA
caggacacaaggcctgttactagcactcacatggaacaaatggcccagatctggccgcactcgag

SEQ ID NO: 3 - RNA, 19 nt, synthetic construct
  source 1..19: mol_type = other RNA
gttttggccactgactgac

SEQ ID NO: 4 - RNA, 177 nt, synthetic construct
  source 1..177: mol_type = other RNA
  misc_feature 34..63: note = up to 20 "n" residues may be deleted
  misc_feature 83..112: note = up to 20 "n" residues may be deleted
ggatcctggaggcttgctgaaggctgtatgctgnnnnnnnnnnnnnnnnnnnnnnnnnnnnnngttttggccactgactgacnnnnnnnnnnnnnnnnnnnnnnnnnnnnnncaggacacaaggcctgttactagcactcacatggaacaaatggcccagatctggccgcactcgag

SEQ ID NO: 5 - RNA, 190 nt, synthetic construct
  source 1..190: mol_type = other RNA
  misc_feature 40..69: note = up to 20 "n" residues may be deleted
  misc_feature 89..118: note = up to 20 "n" residues may be deleted
ggatcctggaggcttgctgaaggctgtatgctgaattcgnnnnnnnnnnnnnnnnnnnnnnnnnnnnnngttttggccactgactgacnnnnnnnnnnnnnnnnnnnnnnnnnnnnnncaccggtcaggacacaaggcctgttactagcactcacatggaacaaatggcccagatctggccgcactcgag

SEQ ID NO: 6 - RNA, 20 nt, synthetic construct
  source 1..20: mol_type = other RNA
tgtggcttctcttaactcct

SEQ ID NO: 7 - RNA, 18 nt, synthetic construct
  source 1..18: mol_type = other RNA
aggagttaagaagccaca

SEQ ID NO: 8 - RNA, 20 nt, synthetic construct
  source 1..20: mol_type = other RNA
tgttgcttctcttaattcct

SEQ ID NO: 9 - RNA, 18 nt, synthetic construct
  source 1..18: mol_type = other RNA
aggaattaagaagcaaca

SEQ ID NO: 10 - RNA, 21 nt, synthetic construct
  source 1..21: mol_type = other RNA
aaatgatcttcaaaagtgccc

SEQ ID NO: 11 - RNA, 19 nt, synthetic construct
  source 1..19: mol_type = other RNA
gcacttttggatcattttc

SEQ ID NO: 12 - RNA, 21 nt, synthetic construct
  source 1..21: mol_type = other RNA
aaaatgatcttcaaaagtgcc

SEQ ID NO: 13 - RNA, 19 nt, synthetic construct
  source 1..19: mol_type = other RNA
cacttttagatcattttct

SEQ ID NO: 14 - RNA, 21 nt, synthetic construct
  source 1..21: mol_type = other RNA
aggtaatttccaaattcccaa

SEQ ID NO: 15 - RNA, 19 nt, synthetic construct
  source 1..19: mol_type = other RNA
gggaatttgaattacctat

SEQ ID NO: 16 - RNA, 21 nt, synthetic construct
  source 1..21: mol_type = other RNA
taggtaatttccaaattccca

SEQ ID NO: 17 - RNA, 19 nt, synthetic construct
  source 1..19: mol_type = other RNA
ggaatttggattacctatg

SEQ ID NO: 18 - RNA, 21 nt, synthetic construct
  source 1..21: mol_type = other RNA
ataggtaatttccaaattccc

SEQ ID NO: 19 - RNA, 19 nt, synthetic construct
  source 1..19: mol_type = other RNA
gaatttggattacctatgt

SEQ ID NO: 20 - RNA, 21 nt, synthetic construct
  source 1..21: mol_type = other RNA
taattcctctgcacataggta

SEQ ID NO: 21 - RNA, 19 nt, synthetic construct
  source 1..19: mol_type = other RNA
cctatgtgcaggaattatg

SEQ ID NO: 22 - RNA, 21 nt, synthetic construct
  source 1..21: mol_type = other RNA
ttaagaaggaaagatcataat

SEQ ID NO: 23 - RNA, 19 nt, synthetic construct
  source 1..19: mol_type = other RNA
tatgatctccttcttaaag

SEQ ID NO: 24 - RNA, 21 nt, synthetic construct
  source 1..21: mol_type = other RNA
tttaagaaggaaagatcataa

SEQ ID NO: 25 - RNA, 18 nt, synthetic construct
  source 1..18: mol_type = other RNA
atgatctcttcttaaaga

SEQ ID NO: 26 - RNA, 21 nt, synthetic construct
  source 1..21: mol_type = other RNA
tctttaagaaggaaagatcat

SEQ ID NO: 27 - RNA, 18 nt, synthetic construct
  source 1..18: mol_type = other RNA
gatctttccttaaagacc

SEQ ID NO: 28 - RNA, 21 nt, synthetic construct
  source 1..21: mol_type = other RNA
gttttccaaaggaattcgctc

SEQ ID NO: 29 - RNA, 18 nt, synthetic construct
  source 1..18: mol_type = other RNA
gcgaattttggaaaacct

SEQ ID NO: 30 - RNA, 21 nt, synthetic construct
  source 1..21: mol_type = other RNA
gcaaatacacaaagaaagccc

SEQ ID NO: 31 - RNA, 19 nt, synthetic construct
  source 1..19: mol_type = other RNA
gggctttctgtgtatttgc

SEQ ID NO: 32 - RNA, 21 nt, synthetic construct
  source 1..21: mol_type = other RNA
tttatattcagtcattttcag

SEQ ID NO: 33 - RNA, 18 nt, synthetic construct
  source 1..18: mol_type = other RNA
gaaaatggaatataaact

SEQ ID NO: 34 - RNA, 21 nt, synthetic construct
  source 1..21: mol_type = other RNA
ttctgaattagctgtatcgtc

SEQ ID NO: 35 - RNA, 19 nt, synthetic construct
  source 1..19: mol_type = other RNA
cgatacagaattcagaatc

SEQ ID NO: 36 - RNA, 21 nt, synthetic construct
  source 1..21: mol_type = other RNA
tattgttggatcatattcgtc

SEQ ID NO: 37 - RNA, 19 nt, synthetic construct
  source 1..19: mol_type = other RNA
cgaatatgccaacaataga

SEQ ID NO: 38 - RNA, 21 nt, synthetic construct
  source 1..21: mol_type = other RNA
ttatttatggcaaatacacaa

SEQ ID NO: 39 - RNA, 19 nt, synthetic construct
  source 1..19: mol_type = other RNA
gtgtatttcataaataata

SEQ ID NO: 40 - RNA, 21 nt, synthetic construct
  source 1..21: mol_type = other RNA
tattatttatggcaaatacac

SEQ ID NO: 41 - RNA, 19 nt, synthetic construct
  source 1..19: mol_type = other RNA
gtatttgctaaataatact

SEQ ID NO: 42 - RNA, 21 nt, synthetic construct
  source 1..21: mol_type = other RNA
atatcttcaaatgatttagta

SEQ ID NO: 43 - RNA, 18 nt, synthetic construct
  source 1..18: mol_type = other RNA
ctaaatcagaagatattc

SEQ ID NO: 44 - RNA, 21 nt, synthetic construct
  source 1..21: mol_type = other RNA
taactcttttaatttgttctc

SEQ ID NO: 45 - RNA, 19 nt, synthetic construct
  source 1..19: mol_type = other RNA
gaacaaattaagagttaag

SEQ ID NO: 46 - RNA, 21 nt, synthetic construct
  source 1..21: mol_type = other RNA
ataacttcttgctaagtcctg

SEQ ID NO: 47 - RNA, 19 nt, synthetic construct
  source 1..19: mol_type = other RNA
ggacttagcgaagttatgg

SEQ ID NO: 48 - RNA, 21 nt, synthetic construct
  source 1..21: mol_type = other RNA
tttcaatctgtattgtcggat

SEQ ID NO: 49 - RNA, 19 nt, synthetic construct
  source 1..19: mol_type = other RNA
ccgacaatacattgaaaaa

SEQ ID NO: 50 - RNA, 21 nt, synthetic construct
  source 1..21: mol_type = other RNA
ttttcaatctgtattgtcgga

SEQ ID NO: 51 - RNA, 19 nt, synthetic construct
  source 1..19: mol_type = other RNA
cgacaatacattgaaaaaa